European Patent Application EP 4 180 519 A1, published May 17, 2023. Title: TRANSGENIC T CELL AND CHIMERIC ANTIGEN RECEPTOR T CELL COMPOSITIONS AND RELATED METHODS. Applicant: Memorial Sloan Kettering Cancer Center. The sequence listing filed with the application follows.

SEQUENCE LISTING (41 sequences)

SEQ ID NO: 1 - protein, 407 aa, Moloney murine leukemia virus
ENSSPYTSEHFHYTVTDIKDLTKLGAIYDKTKKYWVYQGKPVMPDQFTFELLDFLHQLTHLSFSKMKALLERSHSPYYMLNRDRTLKNITETCKACAQVNASKSAVKQGTRVRGHRPGTHWEIDFTEIKPGLYGYKYLLVFIDTFSGWIEAFPTKKETAKVVTKKLLEEIFPRFGMPQVLGTDNGPAFVSKVSQTVADLLGIDWKLHCAYRPQSSGQVERMNRTIKETLTKLTLATGSRDWVLLLPLALYRARNTPGPHGLTPYEILYGAPPPLVNFPDPDMTRVTNSPSLQAHLQALYLVQHEVWRPLAAAYQEQLDRPVVPHPYRVGDTVWVRRHQTKNLEPRWKGPYTVLLTTPTALKVDGIAAWIHAAHVKAADPGGGPSSRLTWRVQRSQNPLKIRLTREAP

SEQ ID NO: 2 - protein, 407 aa, synthetic construct
  source 1..407: note = Synthetic polypeptide
ENSSPYTSEHFHYTVTDIKDLTKLGAIYDKTKKYWVYQGKPVMPDQFTFELLDFLHQLTHLSFSKMKALLERSHSPYYMLNRDRTLKNITETCKACAQVNASKSAVKQGTRVRGHRPGTHWEIAFTEIKPGLYGYKYLLVFIDTFSGWIEAFPTKKETAKVVTKKLLEEIFPRFGMPQVLGTDNGPAFVSKVSQTVADLLGIDWKLHCAYRPQSSGQVERMNRTIKETLTKLTLATGSRDWVLLLPLALYRARNTPGPHGLTPYEILYGAPPPLVNFPDPDMTRVTNSPSLQAHLQALYLVQHEVWRPLAAAYQEQLDRPVVPHPYRVGDTVWVRRHQTKNLEPRWKGPYTVLLTTPTALKVDGIAAWIHAAHVKAADPGGGPSSRLTWRVQRSQNPLKIRLTREAP

SEQ ID NO: 3 - protein, 407 aa, synthetic construct
  source 1..407: note = Synthetic polypeptide
ENSSPYTSEHFHYTVTDIKDLTKLGAIYDKTKKYWVYQGKPVMPDQFTFELLDFLHQLTHLSFSKMKALLERSHSPYYMLNRDRTLKNITETCKACAQVNASKSAVKQGTRVRGHRPGTHWEIEFTEIKPGLYGYKYLLVFIDTFSGWIEAFPTKKETAKVVTKKLLEEIFPRFGMPQVLGTDNGPAFVSKVSQTVADLLGIDWKLHCAYRPQSSGQVERMNRTIKETLTKLTLATGSRDWVLLLPLALYRARNTPGPHGLTPYEILYGAPPPLVNFPDPDMTRVTNSPSLQAHLQALYLVQHEVWRPLAAAYQEQLDRPVVPHPYRVGDTVWVRRHQTKNLEPRWKGPYTVLLTTPTALKVDGIAAWIHAAHVKAADPGGGPSSRLTWRVQRSQNPLKIRLTREAP

SEQ ID NO: 4 - protein, 407 aa, synthetic construct
  source 1..407: note = Synthetic polypeptide
ENSSPYTSEHFHYTVTDIKDLTKLGAIYDKTKKYWVYQGKPVMPDQFTFELLDFLHQLTHLSFSKMKALLERSHSPYYMLNRDRTLKNITETCKACAQVNASKSAVKQGTRVRGHRPGTHWEINFTEIKPGLYGYKYLLVFIDTFSGWIEAFPTKKETAKVVTKKLLEEIFPRFGMPQVLGTDNGPAFVSKVSQTVADLLGIDWKLHCAYRPQSSGQVERMNRTIKETLTKLTLATGSRDWVLLLPLALYRARNTPGPHGLTPYEILYGAPPPLVNFPDPDMTRVTNSPSLQAHLQALYLVQHEVWRPLAAAYQEQLDRPVVPHPYRVGDTVWVRRHQTKNLEPRWKGPYTVLLTTPTALKVDGIAAWIHAAHVKAADPGGGPSSRLTWRVQRSQNPLKIRLTREAP

SEQ ID NO: 5 - protein, 407 aa, synthetic construct
  source 1..407: note = Synthetic polypeptide
ENSSPYTSEHFHYTVTDIKDLTKLGAIYDKTKKYWVYQGKPVMPDQFTFELLDFLHQLTHLSFSKMKALLERSHSPYYMLNRDRTLKNITETCKACAQVNASKSAVKQGTRVRGHRPGTHWEIVFTEIKPGLYGYKYLLVFIDTFSGWIEAFPTKKETAKVVTKKLLEEIFPRFGMPQVLGTDNGPAFVSKVSQTVADLLGIDWKLHCAYRPQSSGQVERMNRTIKETLTKLTLATGSRDWVLLLPLALYRARNTPGPHGLTPYEILYGAPPPLVNFPDPDMTRVTNSPSLQAHLQALYLVQHEVWRPLAAAYQEQLDRPVVPHPYRVGDTVWVRRHQTKNLEPRWKGPYTVLLTTPTALKVDGIAAWIHAAHVKAADPGGGPSSRLTWRVQRSQNPLKIRLTREAP

SEQ ID NO: 6 - protein, 407 aa, synthetic construct
  source 1..407: note = Synthetic polypeptide
ENSSPYTSEHFHYTVTDIKDLTKLGAIYDKTKKYWVYQGKPVMPDQFTFELLDFLHQLTHLSFSKMKALLERSHSPYYMLNRDRTLKNITETCKACAQVNASKSAVKQGTRVRGHRPGTHWEIDFTEIKPGLYGYKYLLVFIDTFSGWIEAFPTKKETAKVVTKKLLEEIFPRFGMPQVLGTANGPAFVSKVSQTVADLLGIDWKLHCAYRPQSSGQVERMNRTIKETLTKLTLATGSRDWVLLLPLALYRARNTPGPHGLTPYEILYGAPPPLVNFPDPDMTRVTNSPSLQAHLQALYLVQHEVWRPLAAAYQEQLDRPVVPHPYRVGDTVWVRRHQTKNLEPRWKGPYTVLLTTPTALKVDGIAAWIHAAHVKAADPGGGPSSRLTWRVQRSQNPLKIRLTREAP

SEQ ID NO: 7 - protein, 407 aa, synthetic construct
  source 1..407: note = Synthetic polypeptide
ENSSPYTSEHFHYTVTDIKDLTKLGAIYDKTKKYWVYQGKPVMPDQFTFELLDFLHQLTHLSFSKMKALLERSHSPYYMLNRDRTLKNITETCKACAQVNASKSAVKQGTRVRGHRPGTHWEIDFTEIKPGLYGYKYLLVFIDTFSGWIEAFPTKKETAKVVTKKLLEEIFPRFGMPQVLGTNNGPAFVSKVSQTVADLLGIDWKLHCAYRPQSSGQVERMNRTIKETLTKLTLATGSRDWVLLLPLALYRARNTPGPHGLTPYEILYGAPPPLVNFPDPDMTRVTNSPSLQAHLQALYLVQHEVWRPLAAAYQEQLDRPVVPHPYRVGDTVWVRRHQTKNLEPRWKGPYTVLLTTPTALKVDGIAAWIHAAHVKAADPGGGPSSRLTWRVQRSQNPLKIRLTREAP

SEQ ID NO: 8 - protein, 407 aa, synthetic construct
  source 1..407: note = Synthetic polypeptide
ENSSPYTSEHFHYTVTDIKDLTKLGAIYDKTKKYWVYQGKPVMPDQFTFELLDFLHQLTHLSFSKMKALLERSHSPYYMLNRDRTLKNITETCKACAQVNASKSAVKQGTRVRGHRPGTHWEIAFTEIKPGLYGYKYLLVFIDTFSGWIEAFPTKKETAKVVTKKLLEEIFPRFGMPQVLGTANGPAFVSKVSQTVADLLGIDWKLHCAYRPQSSGQVERMNRTIKETLTKLTLATGSRDWVLLLPLALYRARNTPGPHGLTPYEILYGAPPPLVNFPDPDMTRVTNSPSLQAHLQALYLVQHEVWRPLAAAYQEQLDRPVVPHPYRVGDTVWVRRHQTKNLEPRWKGPYTVLLTTPTALKVDGIAAWIHAAHVKAADPGGGPSSRLTWRVQRSQNPLKIRLTREAP

SEQ ID NO: 9 - protein, 407 aa, synthetic construct
  source 1..407: note = Synthetic polypeptide
ENSSPYTSEHFHYTVTDIKDLTKLGAIYDKTKKYWVYQGKPVMPDQFTFELLDFLHQLTHLSFSKMKALLERSHSPYYMLNRDRTLKNITETCKACAQVNASKSAVKQGTRVRGHRPGTHWEIAFTEIKPGLYGYKYLLVFIDTFSGWIEAFPTKKETAKVVTKKLLEEIFPRFGMPQVLGTNNGPAFVSKVSQTVADLLGIDWKLHCAYRPQSSGQVERMNRTIKETLTKLTLATGSRDWVLLLPLALYRARNTPGPHGLTPYEILYGAPPPLVNFPDPDMTRVTNSPSLQAHLQALYLVQHEVWRPLAAAYQEQLDRPVVPHPYRVGDTVWVRRHQTKNLEPRWKGPYTVLLTTPTALKVDGIAAWIHAAHVKAADPGGGPSSRLTWRVQRSQNPLKIRLTREAP

SEQ ID NO: 10 - protein, 407 aa, synthetic construct
  source 1..407: note = Synthetic polypeptide
ENSSPYTSEHFHYTVTDIKDLTKLGAIYDKTKKYWVYQGKPVMPDQFTFELLDFLHQLTHLSFSKMKALLERSHSPYYMLNRDRTLKNITETCKACAQVNASKSAVKQGTRVRGHRPGTHWEIEFTEIKPGLYGYKYLLVFIDTFSGWIEAFPTKKETAKVVTKKLLEEIFPRFGMPQVLGTANGPAFVSKVSQTVADLLGIDWKLHCAYRPQSSGQVERMNRTIKETLTKLTLATGSRDWVLLLPLALYRARNTPGPHGLTPYEILYGAPPPLVNFPDPDMTRVTNSPSLQAHLQALYLVQHEVWRPLAAAYQEQLDRPVVPHPYRVGDTVWVRRHQTKNLEPRWKGPYTVLLTTPTALKVDGIAAWIHAAHVKAADPGGGPSSRLTWRVQRSQNPLKIRLTREAP

SEQ ID NO: 11 - protein, 407 aa, synthetic construct
  source 1..407: note = Synthetic polypeptide
ENSSPYTSEHFHYTVTDIKDLTKLGAIYDKTKKYWVYQGKPVMPDQFTFELLDFLHQLTHLSFSKMKALLERSHSPYYMLNRDRTLKNITETCKACAQVNASKSAVKQGTRVRGHRPGTHWEIEFTEIKPGLYGYKYLLVFIDTFSGWIEAFPTKKETAKVVTKKLLEEIFPRFGMPQVLGTNNGPAFVSKVSQTVADLLGIDWKLHCAYRPQSSGQVERMNRTIKETLTKLTLATGSRDWVLLLPLALYRARNTPGPHGLTPYEILYGAPPPLVNFPDPDMTRVTNSPSLQAHLQALYLVQHEVWRPLAAAYQEQLDRPVVPHPYRVGDTVWVRRHQTKNLEPRWKGPYTVLLTTPTALKVDGIAAWIHAAHVKAADPGGGPSSRLTWRVQRSQNPLKIRLTREAP

SEQ ID NO: 12 - protein, 407 aa, synthetic construct
  source 1..407: note = Synthetic polypeptide
ENSSPYTSEHFHYTVTDIKDLTKLGAIYDKTKKYWVYQGKPVMPDQFTFELLDFLHQLTHLSFSKMKALLERSHSPYYMLNRDRTLKNITETCKACAQVNASKSAVKQGTRVRGHRPGTHWEINFTEIKPGLYGYKYLLVFIDTFSGWIEAFPTKKETAKVVTKKLLEEIFPRFGMPQVLGTANGPAFVSKVSQTVADLLGIDWKLHCAYRPQSSGQVERMNRTIKETLTKLTLATGSRDWVLLLPLALYRARNTPGPHGLTPYEILYGAPPPLVNFPDPDMTRVTNSPSLQAHLQALYLVQHEVWRPLAAAYQEQLDRPVVPHPYRVGDTVWVRRHQTKNLEPRWKGPYTVLLTTPTALKVDGIAAWIHAAHVKAADPGGGPSSRLTWRVQRSQNPLKIRLTREAP

SEQ ID NO: 13 - protein, 407 aa, synthetic construct
  source 1..407: note = Synthetic polypeptide
ENSSPYTSEHFHYTVTDIKDLTKLGAIYDKTKKYWVYQGKPVMPDQFTFELLDFLHQLTHLSFSKMKALLERSHSPYYMLNRDRTLKNITETCKACAQVNASKSAVKQGTRVRGHRPGTHWEINFTEIKPGLYGYKYLLVFIDTFSGWIEAFPTKKETAKVVTKKLLEEIFPRFGMPQVLGTNNGPAFVSKVSQTVADLLGIDWKLHCAYRPQSSGQVERMNRTIKETLTKLTLATGSRDWVLLLPLALYRARNTPGPHGLTPYEILYGAPPPLVNFPDPDMTRVTNSPSLQAHLQALYLVQHEVWRPLAAAYQEQLDRPVVPHPYRVGDTVWVRRHQTKNLEPRWKGPYTVLLTTPTALKVDGIAAWIHAAHVKAADPGGGPSSRLTWRVQRSQNPLKIRLTREAP

SEQ ID NO: 14 - protein, 407 aa, synthetic construct
  source 1..407: note = Synthetic polypeptide
ENSSPYTSEHFHYTVTDIKDLTKLGAIYDKTKKYWVYQGKPVMPDQFTFELLDFLHQLTHLSFSKMKALLERSHSPYYMLNRDRTLKNITETCKACAQVNASKSAVKQGTRVRGHRPGTHWEIVFTEIKPGLYGYKYLLVFIDTFSGWIEAFPTKKETAKVVTKKLLEEIFPRFGMPQVLGTANGPAFVSKVSQTVADLLGIDWKLHCAYRPQSSGQVERMNRTIKETLTKLTLATGSRDWVLLLPLALYRARNTPGPHGLTPYEILYGAPPPLVNFPDPDMTRVTNSPSLQAHLQALYLVQHEVWRPLAAAYQEQLDRPVVPHPYRVGDTVWVRRHQTKNLEPRWKGPYTVLLTTPTALKVDGIAAWIHAAHVKAADPGGGPSSRLTWRVQRSQNPLKIRLTREAP

SEQ ID NO: 15 - protein, 407 aa, synthetic construct
  source 1..407: note = Synthetic polypeptide
ENSSPYTSEHFHYTVTDIKDLTKLGAIYDKTKKYWVYQGKPVMPDQFTFELLDFLHQLTHLSFSKMKALLERSHSPYYMLNRDRTLKNITETCKACAQVNASKSAVKQGTRVRGHRPGTHWEIVFTEIKPGLYGYKYLLVFIDTFSGWIEAFPTKKETAKVVTKKLLEEIFPRFGMPQVLGTNNGPAFVSKVSQTVADLLGIDWKLHCAYRPQSSGQVERMNRTIKETLTKLTLATGSRDWVLLLPLALYRARNTPGPHGLTPYEILYGAPPPLVNFPDPDMTRVTNSPSLQAHLQALYLVQHEVWRPLAAAYQEQLDRPVVPHPYRVGDTVWVRRHQTKNLEPRWKGPYTVLLTTPTALKVDGIAAWIHAAHVKAADPGGGPSSRLTWRVQRSQNPLKIRLTREAP

SEQ ID NO: 16 - protein, 164 aa, Homo sapiens
MKWKALFTAAILQAQLPITEAQSFGLLDPKLCYLLDGILFIYGVILTALFLRVKFSRSADAPAYQQGQNQLYNELNLGRREEYDVLDKRRGRDPEMGGKPQRRKNPQEGLYNELQKDKMAEAYSEIGMKGERRRGKGHDGLYQGLSTATKDTYDALHMQALPPR

SEQ ID NO: 17 - protein, 220 aa, Homo sapiens
MLRLLLALNLFPSIQVTGNKILVKQSPMLVAYDNAVNLSCKYSYNLFSREFRASLHKGLDSAVEVCVVYGNYSQQLQVYSKTGFNCDGKLGNESVTFYLQNLYVNQTDIYFCKIEVMYPPPYLDNEKSNGTIIHVKGKHLCPSPLFPGPSKPFWVLVVVGGVLACYSLLVTVAFIIFWVRSKRSRLLHSDYMNMTPRRPGPTRKHYQPYAPPRDFAAYRS

SEQ ID NO: 18 - protein, 255 aa, Homo sapiens
MGNSCYNIVATLLLVLNFERTRSLQDPCSNCPAGTFCDNNRNQICSPCPPNSFSSAGGQRTCDICRQCKGVFRTRKECSSTSNAECDCTPGFHCLGAGCSMCEQDCKQGQELTKKGCKDCCFGTFNDQKRGICRPWTNCSLDGKSVLVNGTKERDVVCGPSPADLSPGASSVTPPAPAREPGHSPQIISFFLALTSTALLFLLFFLTLRFSVVKRGRKKLLYIFKQPFMRPVQTTQEEDGCSCRFPEEEEGGCEL

SEQ ID NO: 19 - protein, 277 aa, Homo sapiens
MCVGARRLGRGPCAALLLLGLGLSTVTGLHCVGDTYPSNDRCCHECRPGNGMVSRCSRSQNTVCRPCGPGFYNDVVSSKPCKPCTWCNLRSGSERKQLCTATQDTVCRCRAGTQPLDSYKPGVDCAPCPPGHFSPGDNQACKPWTNCTLAGKHTLQPASNSSDAICEDRDPPATQPQETQGPPARPITVQPTEAWPRTSQGPSTRPVEVPGGRAVAAILGLGLVLGLLGPLAILLALYLLRRDQRLPPDAHKPPGGGSFRTPIQEEQADAHSTLAKI

SEQ ID NO: 20 - protein, 199 aa, Homo sapiens
MKSGLWYFFLFCLRIKVLTGEINGSANYEMFIFHNGGVQILCKYPDIVQQFKMQLLKGGQILCDLTKTKGSGNTVSIKSLKFCHSQLSNNSVSFFLYNLDHSHANYYFCNLSIFDPPPFKVTLTGGYLHIYESQLCCQLKFWLPIGCAAFVVVCILGCILICWLTKKKYSSSVHDPNGEYMFMRAVNTAKKSRLTDVTL

SEQ ID NO: 21 - protein, 93 aa, Homo sapiens
MIHLGHILFLLLLPVAAAQTTPGERSSLPAFYPGTSGSCSGCGSLSLPLLAGLVAADAVASLLIVGAVFLCARPRRSPAQEDGKVYINMPGRG

SEQ ID NO: 22 - protein, 235 aa, Homo sapiens
MALPVTALLLPLALLLHAARPSQFRVSPLDRTWNLGETVELKCQVLLSNPTSGCSWLFQPRGAAASPTFLLYLSQNKPKAAEGLDTQRFSGKRLGDTFVLTLSDFRRENEGYYFCSALSNSIMYFSHFVPVFLPAKPTTTPAPRPPTPAPTIASQPLSLRPEACRPAAGGAVHTRGLDFACDIYIWAPLAGTCGVLLLSLVITLYCNHRNRRRVCKCPRPVVKSGDKPSLSARYV

SEQ ID NO: 23 - protein, 458 aa, Homo sapiens
MNRGVPFRHLLLVLQLALLPAATQGKKVVLGKKGDTVELTCTASQKKSIQFHWKNSNQIKILGNQGSFLTKGPSKLNDRADSRRSLWDQGNFPLIIKNLKIEDSDTYICEVEDQKEEVQLLVFGLTANSDTHLLQGQSLTLTLESPPGSSPSVQCRSPRGKNIQGGKTLSVSQLELQDSGTWTCTVLQNQKKVEFKIDIVVLAFQKASSIVYKKEGEQVEFSFPLAFTVEKLTGSGELWWQAERASSSKSWITFDLKNKEVSVKRVTQDPKLQMGKKLPLHLTLPQALPQYAGSGNLTLALEAKTGKLHQEVNLVVMRATQLQKNLTCEVWGPTSPKLMLSLKLENKEAKVSKREKAVWVLNPEAGMWQCLLSDSGQVLLESNIKVLPTWSTPVQPMALIVLGGVAGLLLFIGLGIFFCVRCRHRRRQAERMSQIKRLLSEKKTCQCPHRFQKTCSPI

SEQ ID NO: 24 - RNA, 99 nt, synthetic construct
  source 1..99: mol_type = other RNA; note = Synthetic oligonucleotide
cagggttctggatatctgtgttttagagctagaaatagcaagttaaaataaggctagtccgttatcaacttgaaaaagtggcaccgagtcggtgctttt

SEQ ID NO: 25 - DNA, 49 bp, synthetic construct
  source 1..49: mol_type = other DNA; note = Synthetic oligonucleotide
ttgtcccacagatatccagaaccctgaccctgccgtgtaccagctgaga

SEQ ID NO: 26 - RNA, 99 nt, synthetic construct; identical to SEQ ID NO: 24
  source 1..99: mol_type = other RNA; note = Synthetic oligonucleotide

SEQ ID NO: 27 - RNA, 99 nt, synthetic construct
  source 1..99: mol_type = other RNA; note = Synthetic oligonucleotide
ggccacggagcgagacatctttttagagctagaaatagcaagttaaaataaggctagtccgttatcaacttgaaaaagtggcaccgagtcggtgctttt

SEQ ID NO: 28 - DNA, 47 bp, synthetic construct
  source 1..47: mol_type = other DNA; note = Synthetic oligonucleotide
ttagctgtgctcgcgctactctctctttctggcctggaggctatcca

SEQ ID NO: 29 - DNA, 18 bp, synthetic construct
  source 1..18: mol_type = other DNA; note = Synthetic primer
aacccgttgaaccccatt

SEQ ID NO: 30 - DNA, 20 bp, synthetic construct
  source 1..20: mol_type = other DNA; note = Synthetic primer
ccatccaatcggtagtagcg

SEQ ID NO: 31 - DNA, 20 bp, synthetic construct
  source 1..20: mol_type = other DNA; note = Synthetic primer
cgtgcagtctaaagacttgg

SEQ ID NO: 32 - DNA, 20 bp, synthetic construct
  source 1..20: mol_type = other DNA; note = Synthetic primer
ataggggacttggacaaagg

SEQ ID NO: 33 - DNA, 20 bp, synthetic construct
  source 1..20: mol_type = other DNA; note = Synthetic primer
gaaacccagttcattgccgt

SEQ ID NO: 34 - DNA, 20 bp, synthetic construct
  source 1..20: mol_type = other DNA; note = Synthetic primer
ccccaaggaattgacagttg

SEQ ID NO: 35 - DNA, 20 bp, synthetic construct
  source 1..20: mol_type = other DNA; note = Synthetic primer
actggttcccactggatgag

SEQ ID NO: 36 - DNA, 20 bp, synthetic construct
  source 1..20: mol_type = other DNA; note = Synthetic primer
ccacgccatcctctgtaact

SEQ ID NO: 37 - DNA, 20 bp, synthetic construct
  source 1..20: mol_type = other DNA; note = Synthetic primer
cacaaccacactctggagga

SEQ ID NO: 38 - DNA, 20 bp, synthetic construct
  source 1..20: mol_type = other DNA; note = Synthetic primer
ggtttctggtctggatgcct

SEQ ID NO: 39 - DNA, 20 bp, synthetic construct
  source 1..20: mol_type = other DNA; note = Synthetic primer
acaatgagaagagcaatgga

SEQ ID NO: 40 - DNA, 20 bp, synthetic construct
  source 1..20: mol_type = other DNA; note = Synthetic primer
gagattgtcctggtttctgt

SEQ ID NO: 41 - DNA, 80 bp, synthetic construct
  source 1..80: mol_type = other DNA; note = Synthetic oligonucleotide
tcctaaccctgatcctcttgtcccacagatatccagaaccctgaccctgccgtgtaccagctgagagactctaaatccag